European Patent Application EP 4 239 060 A1, published September 6, 2023. Title: Transformed Immune Cells Inducing Chemotaxis for Heterogeneous Immune Cells. Applicant: TSD LIFE SCIENCES. The sequence listing filed with the application follows.

SEQUENCE LISTING (4 sequences)

SEQ ID NO: 1 - protein, 177 aa, Homo sapiens
MFHVSFRYIFGLPPLILVLLPVASSDCDIEGKDGKQYESVLMVSIDQLLDSMKEIGSNCLNNEFNFFKRHICDANKEGMFLFRAARKLRQFLKMNSTGDFDLHLLKVSEGTTILLNCTGQVKGRKPAALGEAQPTKSLEENKSLKEQKKLNDLCFLKRLLQEIKTCWNKILMGTKEH

SEQ ID NO: 2 - protein, 98 aa, Homo sapiens
MALLLALSLLVLWTSPAPTLSGTNDAEDCCLSVTQKPIPGYIVRNFHYLLIKDGCRVPAVVFTTLRGRQLCAPPDQPWVERIIQRLQRTSAKMKRRSS

SEQ ID NO: 3 - DNA, 534 bp, Homo sapiens
atgttccacgtctctttccggtacattttcgggctccccccactgatactggttcttctgccagtcgcatcatctgattgtgatatagagggtaaggacggaaaacaatatgaatctgtactgatggtgtcaatagaccagcttctcgatagcatgaaggaaattggtagtaattgtcttaataatgagttcaacttcttcaaacgccacatatgcgacgccaataaagagggtatgttcttgtttcgcgcggctaggaaactcagacaatttctcaaaatgaactctactggtgacttcgacctccaccttctgaaagtttccgaaggaactaccattcttctgaattgtacaggtcaggtcaaagggcgcaaaccagctgctcttggagaggcccagccaacgaagtcacttgaagaaaataagtctttgaaggaacaaaagaagctgaatgacctgtgctttctcaaaaggctgttgcaggagattaagacctgttggaacaaaatactcatggggaccaaggagcactga

SEQ ID NO: 4 - DNA, 297 bp, Homo sapiens
atggcactgctcctcgccctgagtctcctggtactgtggacatcccctgcgcctacgctctcaggtacaaatgacgccgaagattgctgtctcagtgtaacccagaagcccataccgggttacattgtacggaacttccattatcttctgataaaagacggttgccgagtgcctgccgtggttttcacgacgttgagaggcagacagctgtgcgccccacccgaccagccgtgggtcgagcggatcatacaacgcttgcaaagaacgtccgcgaaaatgaaaaggcgctctagctaa